European Patent Application EP 4 706 686 A1, published March 11, 2026. Title: 스클레로스틴 억제제를 유효성분으로 포함하는 당뇨병성 안질환 예방 또는 치료용 약학적 조성물. Applicant: 중앙대학교 산학협력단. The sequence listing filed with the application follows.

SEQUENCE LISTING (34 sequences)

SEQ ID NO: 1 - DNA, 20 bp, synthetic construct
  source 1..20: mol_type = other DNA
gagcctgtgctactggaagg

SEQ ID NO: 2 - DNA, 19 bp, synthetic construct
  source 1..19: mol_type = other DNA
tgatttccgtggcatcatt

SEQ ID NO: 3 - DNA, 20 bp, synthetic construct
  source 1..20: mol_type = other DNA
ggtgcccgctgctgtctaat

SEQ ID NO: 4 - DNA, 20 bp, synthetic construct
  source 1..20: mol_type = other DNA
tgcaacgcgagtctgtgttt

SEQ ID NO: 5 - DNA, 21 bp, synthetic construct
  source 1..21: mol_type = other DNA
aagctgaggggcagctccagt

SEQ ID NO: 6 - DNA, 21 bp, synthetic construct
  source 1..21: mol_type = other DNA
tctggtaggagacggcgatgc

SEQ ID NO: 7 - DNA, 20 bp, synthetic construct
  source 1..20: mol_type = other DNA
cttcgtgtcctgtatggccc

SEQ ID NO: 8 - DNA, 20 bp, synthetic construct
  source 1..20: mol_type = other DNA
cacattggagtctgctggga

SEQ ID NO: 9 - DNA, 22 bp, synthetic construct
  source 1..22: mol_type = other DNA
gtcaatgttgcccccagagata

SEQ ID NO: 10 - DNA, 20 bp, synthetic construct
  source 1..20: mol_type = other DNA
acaggattttcggagcagga

SEQ ID NO: 11 - DNA, 22 bp, synthetic construct
  source 1..22: mol_type = other DNA
gctctacacctccaatgtgacc

SEQ ID NO: 12 - DNA, 22 bp, synthetic construct
  source 1..22: mol_type = other DNA
ctgccgagatttgagcctcatg

SEQ ID NO: 13 - DNA, 28 bp, synthetic construct
  source 1..28: mol_type = other DNA
cacttatggacaactatgaggtctctgg

SEQ ID NO: 14 - DNA, 32 bp, synthetic construct
  source 1..32: mol_type = other DNA
ctgtcttgtggacaacgcagtggaattttagg

SEQ ID NO: 15 - DNA, 24 bp, synthetic construct
  source 1..24: mol_type = other DNA
ttgctggcagggttgctggtggta

SEQ ID NO: 16 - DNA, 25 bp, synthetic construct
  source 1..25: mol_type = other DNA
catctgcctgctctggtcaatggaa

SEQ ID NO: 17 - DNA, 22 bp, synthetic construct
  source 1..22: mol_type = other DNA
ttgctcaagtgtctgaagcagc

SEQ ID NO: 18 - DNA, 20 bp, synthetic construct
  source 1..20: mol_type = other DNA
cttgctgtagtggtggtcgg

SEQ ID NO: 19 - DNA, 22 bp, synthetic construct
  source 1..22: mol_type = other DNA
ggattcaatgaggagacttgcc

SEQ ID NO: 20 - DNA, 20 bp, synthetic construct
  source 1..20: mol_type = other DNA
gggtcaggggtggttattgc

SEQ ID NO: 21 - DNA, 21 bp, synthetic construct
  source 1..21: mol_type = other DNA
ggctgagactaacccagaaac

SEQ ID NO: 22 - DNA, 21 bp, synthetic construct
  source 1..21: mol_type = other DNA
gaatgaaggtggctgctatga

SEQ ID NO: 23 - DNA, 19 bp, synthetic construct
  source 1..19: mol_type = other DNA
gtgacaatggtggctgctc

SEQ ID NO: 24 - DNA, 20 bp, synthetic construct
  source 1..20: mol_type = other DNA
tccacaggtcagcaggttct

SEQ ID NO: 25 - DNA, 20 bp, synthetic construct
  source 1..20: mol_type = other DNA
tcaatgatcagctccctcag

SEQ ID NO: 26 - DNA, 20 bp, synthetic construct
  source 1..20: mol_type = other DNA
taagtgcctttggtgcttga

SEQ ID NO: 27 - DNA, 20 bp, synthetic construct
  source 1..20: mol_type = other DNA
tctcccattgaaaacatcca

SEQ ID NO: 28 - DNA, 19 bp, synthetic construct
  source 1..19: mol_type = other DNA
ctgtggctccctcagcttc

SEQ ID NO: 29 - DNA, 20 bp, synthetic construct
  source 1..20: mol_type = other DNA
tgttgggccacagtattcct

SEQ ID NO: 30 - DNA, 20 bp, synthetic construct
  source 1..20: mol_type = other DNA
cactcctggatgccaatctt

SEQ ID NO: 31 - DNA, 20 bp, synthetic construct
  source 1..20: mol_type = other DNA
ttaagcccaggagttgcttt

SEQ ID NO: 32 - DNA, 20 bp, synthetic construct
  source 1..20: mol_type = other DNA
caattacaacctgggcgaag

SEQ ID NO: 33 - DNA, 24 bp, synthetic construct
  source 1..24: mol_type = other DNA
gagaaacctgccaagtatgatgac

SEQ ID NO: 34 - DNA, 22 bp, synthetic construct
  source 1..22: mol_type = other DNA
agagtgggagttgctgttgaag